European Patent Application EP 4 310 186 A1, published January 24, 2024. Title: RECOMBINANT MEASLES VIRUS. Applicant: The University of Tokyo. The sequence listing filed with the application follows.

SEQUENCE LISTING (4 sequences)

SEQ ID NO: 1 - DNA, 15894 bp, Artificial Sequence
  Description of Artificial Sequence: Synthesized recombinant measles virus vector
accaaacaaagttgggtaaggatagttcaatcaatgatcatcttctagtgcacttaggattcaagatcctattatcagggacaagagcaggattagggatatccgagatggccacacttttaaggagcttagcattgttcaaaagaaacaaggacaaaccacccattacatcaggatccggtggagccatcagaggaatcaaacacattattatagtaccaatccctggagattcctcaattaccactcgatccagacttctggaccggttggtcaggttaattggaaacccggatgtgagcgggcccaaactaacaggggcactaataggtatattatccttatttgtggagtctccaggtcaattgattcagaggatcaccgatgaccctgacgttagcataaggctgttagaggttgtccagagtgaccagtcacaatctggccttaccttcgcatcaagaggtaccaacatggaggatgaggcggaccaatacttttcacatgatgatccaattagtagtgatcaatccaggttcggatggttcgagaacaaggaaatctcagatattgaagtgcaagaccctgagggattcaacatgattctgggtaccatcctagcccaaatttgggtcttgctcgcaaaggcggttacggccccagacacggcagctgattcggagctaagaaggtggataaagtacacccaacaaagaagggtagttggtgaatttagattggagagaaaatggttggatgtggtgaggaacaggattgccgaggacctctccttacgccgattcatggtcgctctaatcctggatatcaagagaacacccggaaacaaacccaggattgctgaaatgatatgtgacattgatacatatatcgtagaggcaggattagccagttttatcctgactattaagtttgggatagaaactatgtatcctgctcttggactgcatgaatttgctggtgagttatccacacttgagtccttgatgaacctttaccagcaaatgggggaaactgcaccctacatggtaatcctggagaactcaattcagaacaagttcagtgcaggatcataccctctgctctggagctatgccatgggagtaggagtggaacttgaaaactccatgggaggtttgaactttggccgatcttactttgatccagcatattttagattagggcaagagatggtaaggaggtcagctggaaaggtcagttccacattggcatctgaactcggtatcactgccgaggatgcaaggcttgtttcagagattgcaatgcatactactgaggacaagatcagtagagcggttggacccagacaagcccaagtatcatttctacacggtgatcaaagtgagaatgagctaccgagattggggggcaaggaagataggagggtcaaacagagtcgaggagaagccagggagagctacagagaaaccgggcccagcagagcaagtgatgcgagagctgcccatcttccaaccggcacacccctagacattgacactgcatcggagtccagccaagatccgcaggacagtcgaaggtcagctgacgccctgcttaggctgcaagccatggcaggaatctcggaagaacaaggctcagacacggacacccctatagtgtacaatgacagaaatcttctagactagggccggcctgccgaggaccagaacaacatccgcctaccctccatcattgttataaaaaacttaggaaccaggtccacacagccgccagcccatcaaccatccactcccacgattggagcagatggcagaagagcaggcacgccatgtcaaaaacggactggaatgcatccgggctctcaaggccgagcccatcggctcactggccatcgaggaagctatggcagcatggtcagaaatatcagacaacccaggacaggagcgagccacctgcagggaagagaaggcaggcagttcgggtctcagcaaaccatgcctctcagcaattggatcaactgaaggcggtgcacctcgcatccgcggtcagggacctggagagagcgatgacgacgctgaaactttgggaatccccccaagaaatctccaggcatcaagcactgggctacagtgtcattatgtttatgatcacagcggtgaagcggttaagggaatccaagatgctgactctatcatggttcaatcaggccttgatggtgatagcaccctctcaggaggagacaatgaatctgaaaacagcgatgtggatattggcgaacctgataccgagggatatgctatcactgaccggggatctgctcccatctctatggggttcagggcttctgatgttgaaactgcagaaggaggggagatccacgagctcctgagactccaatccagaggcaacaactttccgaagcttgggaaaactctcaatgttcctccgcccccggaccccggtagggccagcacttccgggacacccattaaaaagggcacagacgcgagattagcctcatttggaacggagatcgcgtcttcattgacaggtggtgcaacccaatgtgctcgaaagtcaccctcggaaccatcagggccaggtgcacctgcggggaacgtccccgagtgtgtgagcaatgccgcactgatacaggagtggacacccgaatctggcaccacaatctccccgagatcccagaataatgaagaagggggagaccattatgatgatgagctgttctctgatgtccaagatattaaaacagccttggccaaaatacacgaggataatcagaagataatctccaagctagaatcactgctgttattgaagggagaagttgagtcaattaagaagcagatcaacaggcaaaatatcagcatatccaccctggaaggacacctctcaagcatcatgatcgccattcctggacttgggaaggatcccaacgaccccactgcagatgtcgaaatcaatcccgacttgaaacccatcataggcagagattcaggccgagcactggccgaagttctcaagaaacccgttgccagccgacaactccaaggaatgacaaatggacggaccagttccagaggacagctgctgaaggaatttcagctaaagccgatcgggaaaaagatgagctcagccgtcgggtttgttcctgacaccggccctgcatcacgcagtgtaatccgctccattataaaatccagccggctagaggaggatcggaagcgttacctgatgactctccttgatgatatcaaaggagccaatgatcttgccaagttccaccagatgctggtgaagataataatgaagtagctacagctcaacttacctgccaaccccatgccagtcgacccaactagtacaacctaaatccattataaaaaacttaggagcaaagtgattgcctcccaagttccacaatgacagagatctacgacttcgacaagtcggcatgggacatcaaagggtcgatcgctccgatacaacccaccacctacagtgatggcaggctggtgccccaggtcagagtcatagatcctggtctaggcgacaggaaggatgaatgctttatgtacatgtttctgctgggggttgttgaggacagcgattccctagggcctccaatcgggcgagcatttgggtccctgcccttaggtgttggcagatccacagcaaagcccgaaaaactcctcaaagaggccactgagcttgacatagttgttagacgtacagcagggctcaatgaaaaactggtgttctacaacaacaccccactaactctcctcacaccttggagaaaggtcctaacaacagggagtgtcttcaacgcaaaccaagtgtgcaatgcggttaatctgataccgctcgataccccgcagaggttccgtgttgtttatatgagcatcacccgtctttcggataacgggtattacaccgttcctggaagaatgctggaattcagatcggtcaatgcagtggccttcaacctgctggtgacccttaggattgacaaggcgataggccctgggaagatcatcgacaatacagagcaacttcctgaggcaacatttatggtccacatcgggaacttcaggagaaagaagagtgaagtctactctgccgattattgcaaaatgaaaatcgaaaagatgggcctggtttttgcacttggtgggatagggggcaccagtcttcacattagaagcacaggcaaaatgagcaagactctccatgcacaactcgggttcaagaagaccttatgttacccgctgatggatatcaatgaagaccttaatcgattactctggaggagcagatgcaagatagtaagaatccaggcagttttgcagccatcagttcctcaagaattccgcatttacgacgacgtgatcataaatgatgaccaaggactattcaaagttctgtagaccgtagtgcccagcaatgcccgaaaacgacccccctcacaatgacagccagaaggcccggacaaaaaagccccctccgaaagactccacggaccaagcgagaggccagccagcagccgacggcaagcgcgaacaccaggcggccccagcacagaacagccctgacacaaggccaccaccagccaccccaatctgcatcctcctcgtgggacccccgaggaccaacccccaaggctgcccccgatccaaaccaccaaccgcatccccaccacccccgggaaagaaacccccagcaattggaaggcccctccccctcttcctcaacacaagaactccacaaccgaaccgcacaagcgaccgaggtgacccaaccgcaggcatccgactccctagacagatcctctctccccggcaaactaaacaaaacttagggccaaggaacatacacacccaacagaacccagaccccggcccacggcgccgcgcccccaacccccgacaaccagagggagcccccaaccaatcccgccggctcccccggtgcccacaggcagggacaccaacccccgaacagacccagcacccaaccatcgacaatccaagacgggggggcccccccaaaaaaaggcccccaggggccgacagccagcaccgcgaggaagcccacccaccccacacacgaccacggcaaccaaaccagaacccagaccaccctgggccaccagctcccagactcggccatcaccccgcagaaaggaaaggccacaacccgcgcaccccagccccgatccggcggggagccacccaacccgaaccagcacccaagagcgatccccgaaggacccccgaaccgcaaaggacatcagtatcccacagcctctccaagtcccccggtctcctcctcttctcgaagggaccaaaagatcaatccaccacacccgacgacactcaactccccacccctaaaggagacaccgggaatcccagaatcaagactcatccaatgtccatcatgggtctcaaggtgaacgtctctgccatattcatggcagtactgttaactctccaaacacccaccggtcaaatccattggggcaatctctctaagataggggtggtaggaataggaagtgcaagctacaaagttatgactcgttccagccatcaatcattagtcataaaattaatgcccaatataactctcctcaataactgcacgagggtagagattgcagaatacaggagactactgagaacagttttggaaccaattagagatgcacttaatgcagtgacccagaatataagaccggttcagagtgtagcttcaagtaggagacacaagagatttgcgggagtagtcctggcaggtgcggccctaggcgttgccacagctgctcagataacagccggcattgcacttcaccagtccatgctgaactctcaagccatcgacaatctgagagcgagcctggaaactactaatcaggcaattgaggcaatcagacaagcagggcaggagatgatattggctgttcagggtgtccaagactacatcaataatgagctgataccgtctatgaaccaactatcttgtgatttaatcggccagaagctcgggctcaaattgctcagatactatacagaaatcctgtcattatttggccccagcttacgggaccccatatctgcggagatatctatccaggctttgagctatgcgcttggaggagacatcaataaggtgttagaaaagctcggatacagtggaggtgatttactgggcatcttagagagcagaggaataaaggcccggataactcacgtcgacacagagtcctacttcattgtcctcagtatagcctatccgacgctgtccgagattaagggggtgattgtccaccggctagagggggtctcgtacaacataggctctcaagagtggtataccactgtgcccaagtatgttgcaacccaagggtaccttatctcgaattttgatgagtcatcgtgtactttcatgccagaggggactgtgtgcagccaaaatgccttgtacccgatgagtcctctgctccaagaatgcctccgggggtccaccaagtcctgtgctcgtacactcgtatccgggtcttttgggaaccggttcattttatcacaagggaacctaatagccaattgtgcatcaatcctttgcaagtgttacacaacaggaacgatcattaatcaagaccctgacaagatcctaacatacattgctgccgatcactgcccggtagtcgaggtgaacggcgtgaccatccaagtcgggagcaggaggtatccagacgctgtgtacttgcacagaattgacctcggtcctcccatatcattggagaggttggacgtagggacaaatctggggaatgcaattgctaagttggaggatgccaaggaattgttggagtcatcggaccagatattgaggagtatgaaaggtttatcgagcactagcatagtctacatcctgattgcagtgtgtcttggagggttgatagggatccccgctttaatatgttgctgcagggggcgttgtaacaaaaagggagaacaagttggtatgtcaagaccaggcctaaagcctgatcttacgggaacatcaaaatcctatgtaaggtcgctctgatcctctacaactcttgaaacacaaatgtcccacaagtctcctcttcgtcatcaagcaaccaccgcacccagcatcaagcccacctgaaattatctccggtttccctctggccgaacaatatcggtagttaattaaaacttagggtgcaagatcatccacaatgtcaccacaacgagaccggataaatgccttctacaaagataacccccatcccaagggaagtaggatagtcattaacagagaacatcttatgattgatagaccttatgttttgctggctgttctgtttgtcatgtttctgagcttgatcgggttgctagccattgcaggcattagacttcatcgggcagccatctacaccgcagagatccataaaagcctcagcaccaatctagatgtaactaactcaatcgagcatcaggtcaaggacgtgctgacaccactcttcaaaatcatcggtgatgaagtgggcctgaggacacctcagagattcactgacctagtgaaattcatctctgacaagattaaattccttaatccggatagggagtacgacttcagagatctcacttggtgtatcaacccgccagagagaatcaaattggattatgatcaatactgtgcagatgtggctgctgaagagctcatgaatgcattggtgaactcaactctactggagaccagaacaaccaatcagttcctagctgtctcaaagggaaactgctcagggcccactacaatcagaggtcaattctcaaacatgtcgctgtccctgttagacttgtatttaggtcgaggttacaatgtgtcatctatagtcactatgacatcccagggaatgtatgggggaacttacctagtggaaaagcctaatctgagcagcaaaaggtcagagttgtcacaactgagcatgtaccgagtgtttgaagtaggtgttatcagaaatccgggtttgggggctccggtgttccatatgacaaactatcttgagcaaccagtcagtaatgatctcagcaactgtatggtggctttgggggagctcaaactcgcagccctttgtcacggggaagattctatcacaattccctatcagggatcagggaaaggtgtcagcttccagctcgtcaagctaggtgtctggaaatccccaaccgacatgcaatcctgggtccccttatcaacggatgatccagtgatagacaggctttacctctcatctcacagaggtgttatcgctgacaaccaagcaaaatgggctgtcccgacaacacgaacagatgacaagttgcgaatggagacatgcttccaacaggcgtgtaagggtaaaatccaagcactctgcgagaatcccgagtgggcaccattgaaggataacaggattccttcatacggggtcttgtctgttgatctgagtctgacagttgagcttaaaatcaaaattgcttcgggattcgggccattgatcacacacggttcagggatggacctatacaaatccaaccacaacaatgtgtattggctgactatcccgccaatgaagaacctagccttaggtgtaatcaacacattggagtggataccgagattcaaggttagtccctacctcttcactgtcccaattaaggaagcaggcggagactgccatgccccaacatacctacctgcggaggtggatggtgatgtcaaactcagttccaatctggtgattctacctggtcaagatctccaatatgttttggcaacctacgatacttccagggttgaacatgctgtggtttattacgtttacagcccaagccgctcattttcttacttttatccttttaggttgcctataaagggggtccccatcgaattacaagtggaatgcttcacatgggaccaaaaactctggtgccgtcacttctgtgtgcttgcggactcagaatctggtggacatatcactcactctgggatggtgggcatgggagtcagctgcacagtcacccgggaagatggaaccaatcgcagatagggctgctagtgaaccaatcacatgatgtcacccagacatcaggcatacccactagtgtgaaatagacatcagaattaagaaaaacgtagggtccaagtggttccccgttatggactcgctatctgtcaaccagatcttataccctgaagttcacctagatagcccgatagttaccaataagatagtagccatcctggagtatgctcgagtccctcacgcttacagcctggaggaccctacactgtgtcagaacatcaagcaccgcctaaaaaacggattttccaaccaaatgattataaacaatgtggaagttgggaatgtcatcaagtccaagcttaggagttatccggcccactctcatattccatatccaaattgtaatcaggatttatttaacatagaagacaaagagtcaacgaggaagatccgtgaactcctcaaaaaggggaattcgctgtactccaaagtcagtgataaggttttccaatgcttaagggacactaactcacggcttggcctaggctccgaattgagggaggacatcaaggagaaagttattaacttgggagtttacatgcacagctcccagtggtttgagccctttctgttttggtttacagtcaagactgagatgaggtcagtgattaaatcacaaacccatacttgccataggaggagacacacacctgtattcttcactggtagttcagttgagttgctaatctctcgtgaccttgttgctataatcagtaaagagtctcaacatgtatattacctgacatttgaactggttttgatgtattgtgatgtcatagaggggaggttaatgacagagaccgctatgactattgatgctaggtatacagagcttctaggaagagtcagatacatgtggaaactgatagatggtttcttccctgcactcgggaatccaacttatcaaattgtagccatgctggagcctctttcacttgcttacctgcagctgagggatataacagtagaactcagaggtgctttccttaaccactgctttactgaaatacatgatgttcttgaccaaaacgggttttctgatgaaggtacttatcatgagttaattgaagctctagattacattttcataactgatgacatacatctgacaggggagattttctcatttttcagaagtttcggccaccccagacttgaagcagtaacggctgctgaaaatgttaggaaatacatgaatcagcctaaagtcattgtgtatgagactctgatgaaaggtcatgccatattttgtggaatcataatcaacggctatcgtgacaggcacggaggcagttggccaccgctgaccctccccctgcatgctgcagacacaatccggaatgctcaagcttcaggtgatgggttaacacatgagcagtgcgttgataactggaaatcttttgctggagtgaaatttggctgctttatgcctcttagcctggatagtgatctgacaatgtacctaaaggacaaggcacttgctgctctccaaagggaatgggattcagtttacccgaaagagttcctgcgttacgaccctcccaagggaaccgggtcacggaggcttgtagatgttttccttaatgattcgagctttgacccatatgatgtgataatgtatgttgtaagtggagcttacctccatgaccctgagttcaacctgtcttacagcctgaaagaaaaggagatcaaggaaacaggtagactttttgctaaaatgacttacaaaatgagggcatgccaagtgattgctgaaaatctaatctcaaacgggattggcaaatattttaaggacaatgggatggccaaggatgagcacgatttgactaaggcactccacactctagctgtctcaggagtccccaaagatctcaaagaaagtcacaggggggggccagtcttaaaaacctactcccgaagcccagtccacacaagtaccaggaacgtgagagcagcaaaagggtttatagggttccctcaagtaattcggcaggaccaagacactgatcatccggagaatatggaagcttacgagacagtcagtgcatttatcacgactgatctcaagaagtactgccttaattggagatatgagaccatcagcttgtttgcacagaggctaaatgagatttacggattgccctcatttttccagtggctgcataagaggcttgagacctctgtcctgtatgtaagtgaccctcattgcccccccgaccttgacgcccatatcccgttatataaagtccccaatgatcaaatcttcattaagtaccctatgggaggtatagaagggtattgtcagaagctgtggaccatcagcaccattccctatctatacctggctgcttatgagagcggagtaaggattgcttcgttagtgcaaggggacaatcagaccatagccgtaacaaaaagggtacccagcacatggccctacaaccttaagaaacgggaagctgctagagtaactagagattactttgtaattcttaggcaaaggctacatgatattggccatcacctcaaggcaaatgagacaattgtttcatcacatttttttgtctattcaaaaggaatatattatgatgggctacttgtgtcccaatcactcaagagcatcgcaagatgtgtattctggtcagagactatagttgatgaaacaagggcagcatgcagtaatattgctacaacaatggctaaaagcatcgagagaggttatgaccgttaccttgcatattccctgaacgtcctaaaagtgatacagcaaattctgatctctcttggcttcacaatcaattcaaccatgacccgggatgtagtcatacccctcctcacaaacaacgacctcttaataaggatggcactgttgcccgctcctattggggggatgaattatctgaatatgagcaggctgtttgtcagaaacatcggtgatccagtaacatcatcaattgctgatctcaagagaatgattctcgcctcactaatgcctgaagagaccctccatcaggtaatgacacaacaaccgggggactcttcattcctagactgggctagcgacccttactcagcaaatcttgtatgtgtccagagcatcactagactcctcaagaacataactgcaaggtttgtcctgatccatagtccaaacccaatgttaaaaggattattccatgatgacagtaaagaagaggacgagggactggcggcattcctcatggacaggcatattatagtacctagggcagctcatgaaatcctggatcatagtgtcacaggggcaagagagtctattgcaggcatgctggataccacaaaaggcttgattcgagccagcatgaggaaggggggtttaacctctcgagtgataaccagattgtccaattatgactatgaacaattcagagcagggatggtgctattgacaggaagaaagagaaatgtcctcattgacaaagagtcatgttcagtgcagctggcgagagctctaagaagccatatgtgggcgaggctagctcgaggacggcctatttacggccttgaggtccctgatgtactagaatctatgcgaggccaccttattcggcgtcatgagacatgtgtcatctgcgagtgtggatcagtcaactacggatggttttttgtcccctcgggttgccaactggatgatattgacaaggaaacatcatccttgagagtcccatatattggttctaccactgatgagagaacagacatgaagcttgccttcgtaagagccccaagtcgatccttgcgatctgctgttagaatagcaacagtgtactcatgggcttacggtgatgatgatagctcttggaacgaagcctggttgttggctaggcaaagggccaatgtgagcctggaggagctaagggtgatcactcccatctcaacttcgactaatttagcgcataggttgagggatcgtagcactcaagtgaaatactcaggtacatcccttgtccgagtggcgaggtataccacaatctccaacgacaatctctcatttgtcatatcagataagaaggttgatactaactttatataccaacaaggaatgcttctagggttgggtgttttagaaacattgtttcgactcgagaaagataccggatcatctaacacggtattacatcttcacgtcgaaacagattgttgcgtgatcccgatgatagatcatcccaggatacccagctcccgcaagctagagctgagggcagagctatgtaccaacccattgatatatgataatgcacctttaattgacagagatgcaacaaggctatacacccagagccataggaggcaccttgtggaatttgttacatggtccacaccccaactatatcacattttagctaagtccacagcactatctatgattgacctggtaacaaaatttgagaaggaccatatgaatgaaatttcagctctcataggggatgacgatatcaatagtttcataactgagtttctgctcatagagccaagattattcactatctacttgggccagtgtgcggccatcaattgggcatttgatgtacattatcatagaccatcagggaaatatcagatgggtgagctgttgtcatcgttcctttctagaatgagcaaaggagtgtttaaggtgcttgtcaatgctctaagccacccaaagatctacaagaaattctggcattgtggtattatagagcctatccatggtccttcacttgatgctcaaaacttgcacacaactgtgtgcaacatggtttacacatgctatatgacctacctcgacctgttgttgaatgaagagttagaagagttcacatttctcttgtgtgaaagcgacgaggatgtagtaccggacagattcgacaacatccaggcaaaacacttatgtgttctggcagatttgtactgtcaaccagggacctgcccaccaattcaaggtctaagaccggtagagaaatgtgcagttctaaccgaccatatcaaggcagaggctatgttatctccagcaggatcttcgtggaacataaatccaattattgtagaccattactcatgctccctgacttatctccggcgaggatcgatcaaacagataagattgagagttgatccaggattcattttcgacgccctcgctgaggtaaatgtcagtcagccaaagatcggcagcaacaacatctcaaatatgagcatcaaggctttcagacccccacacgatgatgttgcaaaattgctcaaagatatcaacacaagcaagcacaatcttcccatttcagggggcaatctcgccaattatgaaatccatgctttccgcagaatcgggttgaactcatctgcttgctacaaagctgttgagatatcaacattaattaggagatgccttgagccaggggaggacggcttgttcttgggtgagggatcgggttctatgttgatcacttataaggagatacttaaactaagcaagtgcttctataatagtggggtttccgccaattctagatctggtcaaagggaattagcaccctatccctccgaagttggccttgtcgaacacagaatgggagtaggtaatattgtcaaagtgctctttaacgggaggcccgaagtcacgtgggtaggcagtgtagattgcttcaatttcatagttagtaatatccctacctctagtgtggggtttatccattcagatatagagaccttgcctgacaaagatactatagagaagctagaggaattggcagccatcttatcgatggctctgctcctgggcaaaataggatcaatactggtgattaagcttatgcctttcagcggggattttgttcagggatttataagttatgtagggtctcattatagagaagtgaaccttgtataccctagatacagcaacttcatatctactgaatcttatttggttatgacagatctcaaggctaaccggctaatgaatcctgaaaagattaagcagcagataattgaatcatctgtgaggacttcacctggacttataggtcacatcctatccattaagcaactaagctgcatacaagcaattgtgggagacgcagttagtagaggtgatatcaatcctactctgaaaaaacttacacctatagagcaggtgctgatcaattgcgggttggcaattaacggacctaagctgtgcaaagaattgatccaccatgatgttgcctcagggcaagatggattgcttaattctatactcatcctctacagggagttggcaagattcaaagacaaccaaagaagtcaacaagggatgttccacgcttaccccgtattggtaagtagcaggcaacgagaacttatatctaggatcacccgcaaattttgggggcacattcttctttactccgggaacagaaagttgataaataagtttatccagaatctcaagtccggctatctgatactagacttacaccagaatatcttcgttaagaatctatccaagtcagagaaacagattattatgacggggggtttgaaacgtgagtgggtttttaaggtaacagtcaaggagaccaaagaatggtataagttagtcggatacagtgccctgattaaggactaattggttgaactccggaaccctaatcctgccctaggtggttaggcattatttgcaatatattaaagaaaactttgaaaatacgaagtttctattcccagctttgtctggt

SEQ ID NO: 2 - DNA, 15894 bp, Measles virus attenuated strain
  Description: cDNA of Measles virus attenuated strain
accaaacaaagttgggtaaggatagttcaatcaatgatcatcttctagtgcacttaggattcaagatcctattatcagggacaagagcaggattagggatatccgagatggccacacttttaaggagcttagcattgttcaaaagaaacaaggacaaaccacccattacatcaggatccggtggagccatcagaggaatcaaacacattattatagtaccaatccctggagattcctcaattaccactcgatccagacttctggaccggttggtcaggttaattggaaacccggatgtgagcgggcccaaactaacaggggcactaataggtatattatccttatttgtggagtctccaggtcaattgattcagaggatcaccgatgaccctgacgttagcataaggctgttagaggttgtccagagtgaccagtcacaatctggccttaccttcgcatcaagaggtaccaacatggaggatgaggcggaccaatacttttcacatgatgatccaattagtagtgatcaatccaggttcggatggttcgagaacaaggaaatctcagatattgaagtgcaagaccctgagggattcaacatgattctgggtaccatcctagcccaaatttgggtcttgctcgcaaaggcggttacggccccagacacggcagctgattcggagctaagaaggtggataaagtacacccaacaaagaagggtagttggtgaatttagattggagagaaaatggttggatgtggtgaggaacaggattgccgaggacctctccttacgccgattcatggtcgctctaatcctggatatcaagagaacacccggaaacaaacccaggattgctgaaatgatatgtgacattgatacatatatcgtagaggcaggattagccagttttatcctgactattaagtttgggatagaaactatgtatcctgctcttggactgcatgaatttgctggtgagttatccacacttgagtccttgatgaacctttaccagcaaatgggggaaactgcaccctacatggtaatcctggagaactcaattcagaacaagttcagtgcaggatcataccctctgctctggagctatgccatgggagtaggagtggaacttgaaaactccatgggaggtttgaactttggccgatcttactttgatccagcatattttagattagggcaagagatggtaaggaggtcagctggaaaggtcagttccacattggcatctgaactcggtatcactgccgaggatgcaaggcttgtttcagagattgcaatgcatactactgaggacaagatcagtagagcggttggacccagacaagcccaagtatcatttctacacggtgatcaaagtgagaatgagctaccgagattggggggcaaggaagataggagggtcaaacagagtcgaggagaagccagggagagctacagagaaaccgggcccagcagagcaagtgatgcgagagctgcccatcttccaaccggcacacccctagacattgacactgcatcggagtccagccaagatccgcaggacagtcgaaggtcagctgacgccctgcttaggctgcaagccatggcaggaatctcggaagaacaaggctcagacacggacacccctatagtgtacaatgacagaaatcttctagactaggtgcgagatgccgaggaccagaacaacatccgcctaccctccatcattgttataaaaaacttaggaaccaggtccacacagccgccagcccatcaaccatccactcccacgattggagcagatggcagaagagcaggcacgccatgtcaaaaacggactggaatgcatccgggctctcaaggccgagcccatcggctcactggccatcgaggaagctatggcagcatggtcagaaatatcagacaacccaggacaggagcgagccacctgcagggaagagaaggcaggcagttcgggtctcagcaaaccatgcctctcagcaattggatcaactgaaggcggtgcacctcgcatccgcggtcagggacctggagagagcgatgacgacgctgaaactttgggaatccccccaagaaatctccaggcatcaagcactgggctacagtgtcattatgtttatgatcacagcggtgaagcggttaagggaatccaagatgctgactctatcatggttcaatcaggccttgatggtgatagcaccctctcaggaggagacaatgaatctgaaaacagcgatgtggatattggcgaacctgataccgagggatatgctatcactgaccggggatctgctcccatctctatggggttcagggcttctgatgttgaaactgcagaaggaggggagatccacgagctcctgagactccaatccagaggcaacaactttccgaagcttgggaaaactctcaatgttcctccgcccccggaccccggtagggccagcacttccgggacacccattaaaaagggcacagacgcgagattagcctcatttggaacggagatcgcgtcttcattgacaggtggtgcaacccaatgtgctcgaaagtcaccctcggaaccatcagggccaggtgcacctgcggggaacgtccccgagtgtgtgagcaatgccgcactgatacaggagtggacacccgaatctggcaccacaatctccccgagatcccagaataatgaagaagggggagaccattatgatgatgagctgttctctgatgtccaagatattaaaacagccttggccaaaatacacgaggataatcagaagataatctccaagctagaatcactgctgttattgaagggagaagttgagtcaattaagaagcagatcaacaggcaaaatatcagcatatccaccctggaaggacacctctcaagcatcatgatcgccattcctggacttgggaaggatcccaacgaccccactgcagatgtcgaaatcaatcccgacttgaaacccatcataggcagagattcaggccgagcactggccgaagttctcaagaaacccgttgccagccgacaactccaaggaatgacaaatggacggaccagttccagaggacagctgctgaaggaatttcagctaaagccgatcgggaaaaagatgagctcagccgtcgggtttgttcctgacaccggccctgcatcacgcagtgtaatccgctccattataaaatccagccggctagaggaggatcggaagcgttacctgatgactctccttgatgatatcaaaggagccaatgatcttgccaagttccaccagatgctggtgaagataataatgaagtagctacagctcaacttacctgccaaccccatgccagtcgacccaactagtacaacctaaatccattataaaaaacttaggagcaaagtgattgcctcccaagttccacaatgacagagatctacgacttcgacaagtcggcatgggacatcaaagggtcgatcgctccgatacaacccaccacctacagtgatggcaggctggtgccccaggtcagagtcatagatcctggtctaggcgacaggaaggatgaatgctttatgtacatgtttctgctgggggttgttgaggacagcgattccctagggcctccaatcgggcgagcatttgggtccctgcccttaggtgttggcagatccacagcaaagcccgaaaaactcctcaaagaggccactgagcttgacatagttgttagacgtacagcagggctcaatgaaaaactggtgttctacaacaacaccccactaactctcctcacaccttggagaaaggtcctaacaacagggagtgtcttcaacgcaaaccaagtgtgcaatgcggttaatctgataccgctcgataccccgcagaggttccgtgttgtttatatgagcatcacccgtctttcggataacgggtattacaccgttcctggaagaatgctggaattcagatcggtcaatgcagtggccttcaacctgctggtgacccttaggattgacaaggcgataggccctgggaagatcatcgacaatacagagcaacttcctgaggcaacatttatggtccacatcgggaacttcaggagaaagaagagtgaagtctactctgccgattattgcaaaatgaaaatcgaaaagatgggcctggtttttgcacttggtgggatagggggcaccagtcttcacattagaagcacaggcaaaatgagcaagactctccatgcacaactcgggttcaagaagaccttatgttacccgctgatggatatcaatgaagaccttaatcgattactctggaggagcagatgcaagatagtaagaatccaggcagttttgcagccatcagttcctcaagaattccgcatttacgacgacgtgatcataaatgatgaccaaggactattcaaagttctgtagaccgtagtgcccagcaatgcccgaaaacgacccccctcacaatgacagccagaaggcccggacaaaaaagccccctccgaaagactccacggaccaagcgagaggccagccagcagccgacggcaagcgcgaacaccaggcggccccagcacagaacagccctgacacaaggccaccaccagccaccccaatctgcatcctcctcgtgggacccccgaggaccaacccccaaggctgcccccgatccaaaccaccaaccgcatccccaccacccccgggaaagaaacccccagcaattggaaggcccctccccctcttcctcaacacaagaactccacaaccgaaccgcacaagcgaccgaggtgacccaaccgcaggcatccgactccctagacagatcctctctccccggcaaactaaacaaaacttagggccaaggaacatacacacccaacagaacccagaccccggcccacggcgccgcgcccccaacccccgacaaccagagggagcccccaaccaatcccgccggctcccccggtgcccacaggcagggacaccaacccccgaacagacccagcacccaaccatcgacaatccaagacgggggggcccccccaaaaaaaggcccccaggggccgacagccagcaccgcgaggaagcccacccaccccacacacgaccacggcaaccaaaccagaacccagaccaccctgggccaccagctcccagactcggccatcaccccgcagaaaggaaaggccacaacccgcgcaccccagccccgatccggcggggagccacccaacccgaaccagcacccaagagcgatccccgaaggacccccgaaccgcaaaggacatcagtatcccacagcctctccaagtcccccggtctcctcctcttctcgaagggaccaaaagatcaatccaccacacccgacgacactcaactccccacccctaaaggagacaccgggaatcccagaatcaagactcatccaatgtccatcatgggtctcaaggtgaacgtctctgccatattcatggcagtactgttaactctccaaacacccaccggtcaaatccattggggcaatctctctaagataggggtggtaggaataggaagtgcaagctacaaagttatgactcgttccagccatcaatcattagtcataaaattaatgcccaatataactctcctcaataactgcacgagggtagagattgcagaatacaggagactactgagaacagttttggaaccaattagagatgcacttaatgcagtgacccagaatataagaccggttcagagtgtagcttcaagtaggagacacaagagatttgcgggagtagtcctggcaggtgcggccctaggcgttgccacagctgctcagataacagccggcattgcacttcaccagtccatgctgaactctcaagccatcgacaatctgagagcgagcctggaaactactaatcaggcaattgaggcaatcagacaagcagggcaggagatgatattggctgttcagggtgtccaagactacatcaataatgagctgataccgtctatgaaccaactatcttgtgatttaatcggccagaagctcgggctcaaattgctcagatactatacagaaatcctgtcattatttggccccagcttacgggaccccatatctgcggagatatctatccaggctttgagctatgcgcttggaggagacatcaataaggtgttagaaaagctcggatacagtggaggtgatttactgggcatcttagagagcagaggaataaaggcccggataactcacgtcgacacagagtcctacttcattgtcctcagtatagcctatccgacgctgtccgagattaagggggtgattgtccaccggctagagggggtctcgtacaacataggctctcaagagtggtataccactgtgcccaagtatgttgcaacccaagggtaccttatctcgaattttgatgagtcatcgtgtactttcatgccagaggggactgtgtgcagccaaaatgccttgtacccgatgagtcctctgctccaagaatgcctccgggggtccaccaagtcctgtgctcgtacactcgtatccgggtcttttgggaaccggttcattttatcacaagggaacctaatagccaattgtgcatcaatcctttgcaagtgttacacaacaggaacgatcattaatcaagaccctgacaagatcctaacatacattgctgccgatcactgcccggtagtcgaggtgaacggcgtgaccatccaagtcgggagcaggaggtatccagacgctgtgtacttgcacagaattgacctcggtcctcccatatcattggagaggttggacgtagggacaaatctggggaatgcaattgctaagttggaggatgccaaggaattgttggagtcatcggaccagatattgaggagtatgaaaggtttatcgagcactagcatagtctacatcctgattgcagtgtgtcttggagggttgatagggatccccgctttaatatgttgctgcagggggcgttgtaacaaaaagggagaacaagttggtatgtcaagaccaggcctaaagcctgatcttacgggaacatcaaaatcctatgtaaggtcgctctgatcctctacaactcttgaaacacaaatgtcccacaagtctcctcttcgtcatcaagcaaccaccgcacccagcatcaagcccacctgaaattatctccggtttccctctggccgaacaatatcggtagttaattaaaacttagggtgcaagatcatccacaatgtcaccacaacgagaccggataaatgccttctacaaagataacccccatcccaagggaagtaggatagtcattaacagagaacatcttatgattgatagaccttatgttttgctggctgttctgtttgtcatgtttctgagcttgatcgggttgctagccattgcaggcattagacttcatcgggcagccatctacaccgcagagatccataaaagcctcagcaccaatctagatgtaactaactcaatcgagcatcaggtcaaggacgtgctgacaccactcttcaaaatcatcggtgatgaagtgggcctgaggacacctcagagattcactgacctagtgaaattcatctctgacaagattaaattccttaatccggatagggagtacgacttcagagatctcacttggtgtatcaacccgccagagagaatcaaattggattatgatcaatactgtgcagatgtggctgctgaagagctcatgaatgcattggtgaactcaactctactggagaccagaacaaccaatcagttcctagctgtctcaaagggaaactgctcagggcccactacaatcagaggtcaattctcaaacatgtcgctgtccctgttagacttgtatttaggtcgaggttacaatgtgtcatctatagtcactatgacatcccagggaatgtatgggggaacttacctagtggaaaagcctaatctgagcagcaaaaggtcagagttgtcacaactgagcatgtaccgagtgtttgaagtaggtgttatcagaaatccgggtttgggggctccggtgttccatatgacaaactatcttgagcaaccagtcagtaatgatctcagcaactgtatggtggctttgggggagctcaaactcgcagccctttgtcacggggaagattctatcacaattccctatcagggatcagggaaaggtgtcagcttccagctcgtcaagctaggtgtctggaaatccccaaccgacatgcaatcctgggtccccttatcaacggatgatccagtgatagacaggctttacctctcatctcacagaggtgttatcgctgacaaccaagcaaaatgggctgtcccgacaacacgaacagatgacaagttgcgaatggagacatgcttccaacaggcgtgtaagggtaaaatccaagcactctgcgagaatcccgagtgggcaccattgaaggataacaggattccttcatacggggtcttgtctgttgatctgagtctgacagttgagcttaaaatcaaaattgcttcgggattcgggccattgatcacacacggttcagggatggacctatacaaatccaaccacaacaatgtgtattggctgactatcccgccaatgaagaacctagccttaggtgtaatcaacacattggagtggataccgagattcaaggttagtccctacctcttcactgtcccaattaaggaagcaggcggagactgccatgccccaacatacctacctgcggaggtggatggtgatgtcaaactcagttccaatctggtgattctacctggtcaagatctccaatatgttttggcaacctacgatacttccagggttgaacatgctgtggtttattacgtttacagcccaagccgctcattttcttacttttatccttttaggttgcctataaagggggtccccatcgaattacaagtggaatgcttcacatgggaccaaaaactctggtgccgtcacttctgtgtgcttgcggactcagaatctggtggacatatcactcactctgggatggtgggcatgggagtcagctgcacagtcacccgggaagatggaaccaatcgcagatagggctgctagtgaaccaatcacatgatgtcacccagacatcaggcatacccactagtgtgaaatagacatcagaattaagaaaaacgtagggtccaagtggttccccgttatggactcgctatctgtcaaccagatcttataccctgaagttcacctagatagcccgatagttaccaataagatagtagccatcctggagtatgctcgagtccctcacgcttacagcctggaggaccctacactgtgtcagaacatcaagcaccgcctaaaaaacggattttccaaccaaatgattataaacaatgtggaagttgggaatgtcatcaagtccaagcttaggagttatccggcccactctcatattccatatccaaattgtaatcaggatttatttaacatagaagacaaagagtcaacgaggaagatccgtgaactcctcaaaaaggggaattcgctgtactccaaagtcagtgataaggttttccaatgcttaagggacactaactcacggcttggcctaggctccgaattgagggaggacatcaaggagaaagttattaacttgggagtttacatgcacagctcccagtggtttgagccctttctgttttggtttacagtcaagactgagatgaggtcagtgattaaatcacaaacccatacttgccataggaggagacacacacctgtattcttcactggtagttcagttgagttgctaatctctcgtgaccttgttgctataatcagtaaagagtctcaacatgtatattacctgacatttgaactggttttgatgtattgtgatgtcatagaggggaggttaatgacagagaccgctatgactattgatgctaggtatacagagcttctaggaagagtcagatacatgtggaaactgatagatggtttcttccctgcactcgggaatccaacttatcaaattgtagccatgctggagcctctttcacttgcttacctgcagctgagggatataacagtagaactcagaggtgctttccttaaccactgctttactgaaatacatgatgttcttgaccaaaacgggttttctgatgaaggtacttatcatgagttaattgaagctctagattacattttcataactgatgacatacatctgacaggggagattttctcatttttcagaagtttcggccaccccagacttgaagcagtaacggctgctgaaaatgttaggaaatacatgaatcagcctaaagtcattgtgtatgagactctgatgaaaggtcatgccatattttgtggaatcataatcaacggctatcgtgacaggcacggaggcagttggccaccgctgaccctccccctgcatgctgcagacacaatccggaatgctcaagcttcaggtgatgggttaacacatgagcagtgcgttgataactggaaatcttttgctggagtgaaatttggctgctttatgcctcttagcctggatagtgatctgacaatgtacctaaaggacaaggcacttgctgctctccaaagggaatgggattcagtttacccgaaagagttcctgcgttacgaccctcccaagggaaccgggtcacggaggcttgtagatgttttccttaatgattcgagctttgacccatatgatgtgataatgtatgttgtaagtggagcttacctccatgaccctgagttcaacctgtcttacagcctgaaagaaaaggagatcaaggaaacaggtagactttttgctaaaatgacttacaaaatgagggcatgccaagtgattgctgaaaatctaatctcaaacgggattggcaaatattttaaggacaatgggatggccaaggatgagcacgatttgactaaggcactccacactctagctgtctcaggagtccccaaagatctcaaagaaagtcacaggggggggccagtcttaaaaacctactcccgaagcccagtccacacaagtaccaggaacgtgagagcagcaaaagggtttatagggttccctcaagtaattcggcaggaccaagacactgatcatccggagaatatggaagcttacgagacagtcagtgcatttatcacgactgatctcaagaagtactgccttaattggagatatgagaccatcagcttgtttgcacagaggctaaatgagatttacggattgccctcatttttccagtggctgcataagaggcttgagacctctgtcctgtatgtaagtgaccctcattgcccccccgaccttgacgcccatatcccgttatataaagtccccaatgatcaaatcttcattaagtaccctatgggaggtatagaagggtattgtcagaagctgtggaccatcagcaccattccctatctatacctggctgcttatgagagcggagtaaggattgcttcgttagtgcaaggggacaatcagaccatagccgtaacaaaaagggtacccagcacatggccctacaaccttaagaaacgggaagctgctagagtaactagagattactttgtaattcttaggcaaaggctacatgatattggccatcacctcaaggcaaatgagacaattgtttcatcacatttttttgtctattcaaaaggaatatattatgatgggctacttgtgtcccaatcactcaagagcatcgcaagatgtgtattctggtcagagactatagttgatgaaacaagggcagcatgcagtaatattgctacaacaatggctaaaagcatcgagagaggttatgaccgttaccttgcatattccctgaacgtcctaaaagtgatacagcaaattctgatctctcttggcttcacaatcaattcaaccatgacccgggatgtagtcatacccctcctcacaaacaacgacctcttaataaggatggcactgttgcccgctcctattggggggatgaattatctgaatatgagcaggctgtttgtcagaaacatcggtgatccagtaacatcatcaattgctgatctcaagagaatgattctcgcctcactaatgcctgaagagaccctccatcaggtaatgacacaacaaccgggggactcttcattcctagactgggctagcgacccttactcagcaaatcttgtatgtgtccagagcatcactagactcctcaagaacataactgcaaggtttgtcctgatccatagtccaaacccaatgttaaaaggattattccatgatgacagtaaagaagaggacgagggactggcggcattcctcatggacaggcatattatagtacctagggcagctcatgaaatcctggatcatagtgtcacaggggcaagagagtctattgcaggcatgctggataccacaaaaggcttgattcgagccagcatgaggaaggggggtttaacctctcgagtgataaccagattgtccaattatgactatgaacaattcagagcagggatggtgctattgacaggaagaaagagaaatgtcctcattgacaaagagtcatgttcagtgcagctggcgagagctctaagaagccatatgtgggcgaggctagctcgaggacggcctatttacggccttgaggtccctgatgtactagaatctatgcgaggccaccttattcggcgtcatgagacatgtgtcatctgcgagtgtggatcagtcaactacggatggttttttgtcccctcgggttgccaactggatgatattgacaaggaaacatcatccttgagagtcccatatattggttctaccactgatgagagaacagacatgaagcttgccttcgtaagagccccaagtcgatccttgcgatctgctgttagaatagcaacagtgtactcatgggcttacggtgatgatgatagctcttggaacgaagcctggttgttggctaggcaaagggccaatgtgagcctggaggagctaagggtgatcactcccatctcaacttcgactaatttagcgcataggttgagggatcgtagcactcaagtgaaatactcaggtacatcccttgtccgagtggcgaggtataccacaatctccaacgacaatctctcatttgtcatatcagataagaaggttgatactaactttatataccaacaaggaatgcttctagggttgggtgttttagaaacattgtttcgactcgagaaagataccggatcatctaacacggtattacatcttcacgtcgaaacagattgttgcgtgatcccgatgatagatcatcccaggatacccagctcccgcaagctagagctgagggcagagctatgtaccaacccattgatatatgataatgcacctttaattgacagagatgcaacaaggctatacacccagagccataggaggcaccttgtggaatttgttacatggtccacaccccaactatatcacattttagctaagtccacagcactatctatgattgacctggtaacaaaatttgagaaggaccatatgaatgaaatttcagctctcataggggatgacgatatcaatagtttcataactgagtttctgctcatagagccaagattattcactatctacttgggccagtgtgcggccatcaattgggcatttgatgtacattatcatagaccatcagggaaatatcagatgggtgagctgttgtcatcgttcctttctagaatgagcaaaggagtgtttaaggtgcttgtcaatgctctaagccacccaaagatctacaagaaattctggcattgtggtattatagagcctatccatggtccttcacttgatgctcaaaacttgcacacaactgtgtgcaacatggtttacacatgctatatgacctacctcgacctgttgttgaatgaagagttagaagagttcacatttctcttgtgtgaaagcgacgaggatgtagtaccggacagattcgacaacatccaggcaaaacacttatgtgttctggcagatttgtactgtcaaccagggacctgcccaccaattcaaggtctaagaccggtagagaaatgtgcagttctaaccgaccatatcaaggcagaggctatgttatctccagcaggatcttcgtggaacataaatccaattattgtagaccattactcatgctccctgacttatctccggcgaggatcgatcaaacagataagattgagagttgatccaggattcattttcgacgccctcgctgaggtaaatgtcagtcagccaaagatcggcagcaacaacatctcaaatatgagcatcaaggctttcagacccccacacgatgatgttgcaaaattgctcaaagatatcaacacaagcaagcacaatcttcccatttcagggggcaatctcgccaattatgaaatccatgctttccgcagaatcgggttgaactcatctgcttgctacaaagctgttgagatatcaacattaattaggagatgccttgagccaggggaggacggcttgttcttgggtgagggatcgggttctatgttgatcacttataaggagatacttaaactaagcaagtgcttctataatagtggggtttccgccaattctagatctggtcaaagggaattagcaccctatccctccgaagttggccttgtcgaacacagaatgggagtaggtaatattgtcaaagtgctctttaacgggaggcccgaagtcacgtgggtaggcagtgtagattgcttcaatttcatagttagtaatatccctacctctagtgtggggtttatccattcagatatagagaccttgcctgacaaagatactatagagaagctagaggaattggcagccatcttatcgatggctctgctcctgggcaaaataggatcaatactggtgattaagcttatgcctttcagcggggattttgttcagggatttataagttatgtagggtctcattatagagaagtgaaccttgtataccctagatacagcaacttcatatctactgaatcttatttggttatgacagatctcaaggctaaccggctaatgaatcctgaaaagattaagcagcagataattgaatcatctgtgaggacttcacctggacttataggtcacatcctatccattaagcaactaagctgcatacaagcaattgtgggagacgcagttagtagaggtgatatcaatcctactctgaaaaaacttacacctatagagcaggtgctgatcaattgcgggttggcaattaacggacctaagctgtgcaaagaattgatccaccatgatgttgcctcagggcaagatggattgcttaattctatactcatcctctacagggagttggcaagattcaaagacaaccaaagaagtcaacaagggatgttccacgcttaccccgtattggtaagtagcaggcaacgagaacttatatctaggatcacccgcaaattttgggggcacattcttctttactccgggaacagaaagttgataaataagtttatccagaatctcaagtccggctatctgatactagacttacaccagaatatcttcgttaagaatctatccaagtcagagaaacagattattatgacggggggtttgaaacgtgagtgggtttttaaggtaacagtcaaggagaccaaagaatggtataagttagtcggatacagtgccctgattaaggactaattggttgaactccggaaccctaatcctgccctaggtggttaggcattatttgcaatatattaaagaaaactttgaaaatacgaagtttctattcccagctttgtctggt

SEQ ID NO: 3 - DNA, 19842 bp, Artificial Sequence
  Description of Artificial Sequence: Synthesized cDNA of recombinant measles virus vaccine for SARS-CoV-2
accaaacaaagttgggtaaggatagttcaatcaatgatcatcttctagtgcacttaggattcaagatcctattatcagggacaagagcaggattagggatatccgagatggccacacttttaaggagcttagcattgttcaaaagaaacaaggacaaaccacccattacatcaggatccggtggagccatcagaggaatcaaacacattattatagtaccaatccctggagattcctcaattaccactcgatccagacttctggaccggttggtcaggttaattggaaacccggatgtgagcgggcccaaactaacaggggcactaataggtatattatccttatttgtggagtctccaggtcaattgattcagaggatcaccgatgaccctgacgttagcataaggctgttagaggttgtccagagtgaccagtcacaatctggccttaccttcgcatcaagaggtaccaacatggaggatgaggcggaccaatacttttcacatgatgatccaattagtagtgatcaatccaggttcggatggttcgagaacaaggaaatctcagatattgaagtgcaagaccctgagggattcaacatgattctgggtaccatcctagcccaaatttgggtcttgctcgcaaaggcggttacggccccagacacggcagctgattcggagctaagaaggtggataaagtacacccaacaaagaagggtagttggtgaatttagattggagagaaaatggttggatgtggtgaggaacaggattgccgaggacctctccttacgccgattcatggtcgctctaatcctggatatcaagagaacacccggaaacaaacccaggattgctgaaatgatatgtgacattgatacatatatcgtagaggcaggattagccagttttatcctgactattaagtttgggatagaaactatgtatcctgctcttggactgcatgaatttgctggtgagttatccacacttgagtccttgatgaacctttaccagcaaatgggggaaactgcaccctacatggtaatcctggagaactcaattcagaacaagttcagtgcaggatcataccctctgctctggagctatgccatgggagtaggagtggaacttgaaaactccatgggaggtttgaactttggccgatcttactttgatccagcatattttagattagggcaagagatggtaaggaggtcagctggaaaggtcagttccacattggcatctgaactcggtatcactgccgaggatgcaaggcttgtttcagagattgcaatgcatactactgaggacaagatcagtagagcggttggacccagacaagcccaagtatcatttctacacggtgatcaaagtgagaatgagctaccgagattggggggcaaggaagataggagggtcaaacagagtcgaggagaagccagggagagctacagagaaaccgggcccagcagagcaagtgatgcgagagctgcccatcttccaaccggcacacccctagacattgacactgcatcggagtccagccaagatccgcaggacagtcgaaggtcagctgacgccctgcttaggctgcaagccatggcaggaatctcggaagaacaaggctcagacacggacacccctatagtgtacaatgacagaaatcttctagactagggccggcctgccgaggaccagaacaacatccgcctaccctccatcattgttataaaaaacttaggaaccaggtccacacagccgccagcccatcaaccatccactcccacgattggagcagatgttcgtctttctggtgctccttcctctggtcagttctcagtgtgtgaatctcaccacaagaacccagttgcctcctgcttataccaacagctttacacggggtgtctattatcccgacaaggtgtttcgcagtagcgtactacactctacacaggacctttttctccccttcttctccaatgtcacttggtttcacgctatccacgtctcaggcacaaatggtaccaagcgctttgataatcccgttctgccctttaatgatggggtatattttgcctcaaccgaaaaatccaacatcatccggggatggatttttgggacaacccttgattccaagactcaaagcctgctgatcgttaacaatgctaccaacgttgtcatcaaagtatgcgagttccagttttgcaatgatccatttctcggcgtgtactaccataagaacaataaatcatggatggaatccgaattccgagtgtactcctctgctaacaactgcacctttgaatacgtatctcagccctttctcatggatctcgaaggaaagcagggaaatttcaagaacctccgggaatttgtcttcaagaatatagacgggtacttcaaaatctactctaagcatacccccatcaacctggtgcgcgacctaccacaaggcttcagtgccctagagcccctggtggacttgcccataggcattaatatcacgagatttcagacattattggccctgcacagaagctatctcacccctggcgattccagtagtggatggaccgctggcgcagccgcctattacgtgggatacttgcagccacgaactttcctactcaagtataatgagaacggaaccataaccgatgcagtagattgtgccttggatcctctttctgagacaaaatgtacactgaagtcgttcacagtggagaaagggatctaccagacaagcaacttcagggttcaaccgactgagtctatcgtcaggtttccaaatataaccaacctttgtccgtttggcgaagtgttcaatgccactagattcgcgtccgtctatgcatggaatcgcaaaaggatttccaactgtgtggccgattacagcgtgttgtacaattcagccagcttcagcacctttaagtgctatggagtgtctccaacgaaactcaacgatctgtgtttcacgaatgtgtacgccgattcattcgtcattcggggagacgaagtcagacagatagccccagggcagacagggaaaattgccgactataactacaaactgccagatgacttcaccggttgcgtgatagcttggaattctaataacctcgacagcaaggttggagggaactacaattatctgtaccggctgttccgtaagtcaaacctgaaaccctttgaacgcgacatctccacagagatttaccaagctggatccaccccttgcaatggggtagagggattcaattgctactttccgctgcagtcttatgggtttcaacccaccaatggagtggggtaccagccctaccgagtggttgtcctgtcctttgaattgttgcatgcccccgcgaccgtgtgtggccccaagaagagtacaaatctcgttaaaaacaagtgcgtaaacttcaactttaacggtttgacggggactggggtgctgacggaatcaaacaagaaattcctgccgttccagcagttcgggagggacattgccgacacaaccgacgctgtcagggatccacagaccctggagatcttggacattacaccttgctccttcggcggcgtgagtgtaatcacacctggaactaacacgagtaaccaggttgccgtcctgtaccaagacgtgaattgcaccgaggttccagttgcgatccacgcggatcagcttactcctacatggcgagtgtatagtacaggcagtaacgtattccagactcgtgccgggtgtttaataggggcagaacacgtgaataacagttatgagtgtgacattccgatcggcgctggtatatgcgcatcataccaaacccagactaactcacctagaagagcccgctccgtggccagccagagcattatcgcctatacgatgagcctgggtgctgagaattccgtagcatattctaacaattccattgctattcctaccaactttaccatctctgttaccactgagattctcccagtgtctatgactaagacatcagtggactgcactatgtatatctgcggcgatagcactgagtgtagcaatttgctcctgcaatatggttcattttgcacccagcttaatagggccctgacaggaattgccgttgagcaggacaagaatactcaggaggtcttcgctcaggttaagcagatctacaagactccgccaattaaggacttcggcggatttaacttcagccagattctgccagacccaagtaagccctccaaaaggtcttttatcgaggatctgctgttcaacaaagtgacacttgccgatgctggctttatcaaacagtatggagactgtctcggtgatatagcagcacgggacctcatctgcgcccagaagtttaacggactgaccgtcctgcctcctcttctgacagacgagatgattgctcagtacacttcggcgctgcttgcaggtactatcacaagcggctggacgtttggtgccggagccgcgctccaaattccattcgcaatgcagatggcttatagattcaacggcataggtgtcacccagaacgtgctgtacgaaaaccagaagctcatagcgaaccagtttaactccgccatagggaaaatccaggattcgctctccagtacagcatccgcattagggaaactgcaggacgttgtgaatcagaacgcccaagctcttaatacactggtgaaacaattgtcatccaatttcggggcaatcagctctgtgcttaatgacatcctctcacggctggataaagtcgaagccgaagttcagattgatcgcttgattactggtcggttacagtcactacagacatatgtgacccagcagctgattcgtgctgccgagattagggcatcggctaacctggcagctactaagatgtccgagtgcgtgcttggccaatcgaaacgcgtggatttctgtggcaaaggctatcatctgatgagcttccctcaaagcgcgccccatggcgtggtgtttctgcacgtgacgtatgtccccgcacaggagaagaatttcacaacagcccccgcaatctgtcacgatggcaaggcacactttcctcgagaaggggttttcgtgagcaatggcacccactggttcgtgacccagaggaacttttatgagccgcaaattatcactacggataatacctttgtgagtggaaactgtgacgtggtgattggaatcgtcaacaatactgtatacgaccccttacaacctgaactggactctttcaaagaggaactagacaagtactttaagaaccatacttctccagacgtcgatttaggagacatttcaggcatcaatgccagcgtggtgaacatccagaaggagatcgatagactgaacgaagtcgctaagaatttaaacgaaagcctaatagacctgcaagagctgggcaaatacgagcagtacattaagtggccatggtacatctggttgggcttcatcgctggccttatcgccattgttatggtcaccatcatgctctgctgcatgacttcttgttgcagttgcttaaaagggtgttgcagctgtggcagctgctgtaagttcgacgaggatgattccgagcccgtgctaaaaggtgttaagctgcattacacgtaataataggccggcctgccgaggaccagaacaacatccgcctaccctccatcattgttataaaaaacttaggaaccaggtccacacagccgccagcccatcaaccatccactcccacgattggagcagatggcagaagagcaggcacgccatgtcaaaaacggactggaatgcatccgggctctcaaggccgagcccatcggctcactggccatcgaggaagctatggcagcatggtcagaaatatcagacaacccaggacaggagcgagccacctgcagggaagagaaggcaggcagttcgggtctcagcaaaccatgcctctcagcaattggatcaactgaaggcggtgcacctcgcatccgcggtcagggacctggagagagcgatgacgacgctgaaactttgggaatccccccaagaaatctccaggcatcaagcactgggctacagtgtcattatgtttatgatcacagcggtgaagcggttaagggaatccaagatgctgactctatcatggttcaatcaggccttgatggtgatagcaccctctcaggaggagacaatgaatctgaaaacagcgatgtggatattggcgaacctgataccgagggatatgctatcactgaccggggatctgctcccatctctatggggttcagggcttctgatgttgaaactgcagaaggaggggagatccacgagctcctgagactccaatccagaggcaacaactttccgaagcttgggaaaactctcaatgttcctccgcccccggaccccggtagggccagcacttccgggacacccattaaaaagggcacagacgcgagattagcctcatttggaacggagatcgcgtcttcattgacaggtggtgcaacccaatgtgctcgaaagtcaccctcggaaccatcagggccaggtgcacctgcggggaacgtccccgagtgtgtgagcaatgccgcactgatacaggagtggacacccgaatctggcaccacaatctccccgagatcccagaataatgaagaagggggagaccattatgatgatgagctgttctctgatgtccaagatattaaaacagccttggccaaaatacacgaggataatcagaagataatctccaagctagaatcactgctgttattgaagggagaagttgagtcaattaagaagcagatcaacaggcaaaatatcagcatatccaccctggaaggacacctctcaagcatcatgatcgccattcctggacttgggaaggatcccaacgaccccactgcagatgtcgaaatcaatcccgacttgaaacccatcataggcagagattcaggccgagcactggccgaagttctcaagaaacccgttgccagccgacaactccaaggaatgacaaatggacggaccagttccagaggacagctgctgaaggaatttcagctaaagccgatcgggaaaaagatgagctcagccgtcgggtttgttcctgacaccggccctgcatcacgcagtgtaatccgctccattataaaatccagccggctagaggaggatcggaagcgttacctgatgactctccttgatgatatcaaaggagccaatgatcttgccaagttccaccagatgctggtgaagataataatgaagtagctacagctcaacttacctgccaaccccatgccagtcgacccaactagtacaacctaaatccattataaaaaacttaggagcaaagtgattgcctcccaagttccacaatgacagagatctacgacttcgacaagtcggcatgggacatcaaagggtcgatcgctccgatacaacccaccacctacagtgatggcaggctggtgccccaggtcagagtcatagatcctggtctaggcgacaggaaggatgaatgctttatgtacatgtttctgctgggggttgttgaggacagcgattccctagggcctccaatcgggcgagcatttgggtccctgcccttaggtgttggcagatccacagcaaagcccgaaaaactcctcaaagaggccactgagcttgacatagttgttagacgtacagcagggctcaatgaaaaactggtgttctacaacaacaccccactaactctcctcacaccttggagaaaggtcctaacaacagggagtgtcttcaacgcaaaccaagtgtgcaatgcggttaatctgataccgctcgataccccgcagaggttccgtgttgtttatatgagcatcacccgtctttcggataacgggtattacaccgttcctggaagaatgctggaattcagatcggtcaatgcagtggccttcaacctgctggtgacccttaggattgacaaggcgataggccctgggaagatcatcgacaatacagagcaacttcctgaggcaacatttatggtccacatcgggaacttcaggagaaagaagagtgaagtctactctgccgattattgcaaaatgaaaatcgaaaagatgggcctggtttttgcacttggtgggatagggggcaccagtcttcacattagaagcacaggcaaaatgagcaagactctccatgcacaactcgggttcaagaagaccttatgttacccgctgatggatatcaatgaagaccttaatcgattactctggaggagcagatgcaagatagtaagaatccaggcagttttgcagccatcagttcctcaagaattccgcatttacgacgacgtgatcataaatgatgaccaaggactattcaaagttctgtagaccgtagtgcccagcaatgcccgaaaacgacccccctcacaatgacagccagaaggcccggacaaaaaagccccctccgaaagactccacggaccaagcgagaggccagccagcagccgacggcaagcgcgaacaccaggcggccccagcacagaacagccctgacacaaggccaccaccagccaccccaatctgcatcctcctcgtgggacccccgaggaccaacccccaaggctgcccccgatccaaaccaccaaccgcatccccaccacccccgggaaagaaacccccagcaattggaaggcccctccccctcttcctcaacacaagaactccacaaccgaaccgcacaagcgaccgaggtgacccaaccgcaggcatccgactccctagacagatcctctctccccggcaaactaaacaaaacttagggccaaggaacatacacacccaacagaacccagaccccggcccacggcgccgcgcccccaacccccgacaaccagagggagcccccaaccaatcccgccggctcccccggtgcccacaggcagggacaccaacccccgaacagacccagcacccaaccatcgacaatccaagacgggggggcccccccaaaaaaaggcccccaggggccgacagccagcaccgcgaggaagcccacccaccccacacacgaccacggcaaccaaaccagaacccagaccaccctgggccaccagctcccagactcggccatcaccccgcagaaaggaaaggccacaacccgcgcaccccagccccgatccggcggggagccacccaacccgaaccagcacccaagagcgatccccgaaggacccccgaaccgcaaaggacatcagtatcccacagcctctccaagtcccccggtctcctcctcttctcgaagggaccaaaagatcaatccaccacacccgacgacactcaactccccacccctaaaggagacaccgggaatcccagaatcaagactcatccaatgtccatcatgggtctcaaggtgaacgtctctgccatattcatggcagtactgttaactctccaaacacccaccggtcaaatccattggggcaatctctctaagataggggtggtaggaataggaagtgcaagctacaaagttatgactcgttccagccatcaatcattagtcataaaattaatgcccaatataactctcctcaataactgcacgagggtagagattgcagaatacaggagactactgagaacagttttggaaccaattagagatgcacttaatgcagtgacccagaatataagaccggttcagagtgtagcttcaagtaggagacacaagagatttgcgggagtagtcctggcaggtgcggccctaggcgttgccacagctgctcagataacagccggcattgcacttcaccagtccatgctgaactctcaagccatcgacaatctgagagcgagcctggaaactactaatcaggcaattgaggcaatcagacaagcagggcaggagatgatattggctgttcagggtgtccaagactacatcaataatgagctgataccgtctatgaaccaactatcttgtgatttaatcggccagaagctcgggctcaaattgctcagatactatacagaaatcctgtcattatttggccccagcttacgggaccccatatctgcggagatatctatccaggctttgagctatgcgcttggaggagacatcaataaggtgttagaaaagctcggatacagtggaggtgatttactgggcatcttagagagcagaggaataaaggcccggataactcacgtcgacacagagtcctacttcattgtcctcagtatagcctatccgacgctgtccgagattaagggggtgattgtccaccggctagagggggtctcgtacaacataggctctcaagagtggtataccactgtgcccaagtatgttgcaacccaagggtaccttatctcgaattttgatgagtcatcgtgtactttcatgccagaggggactgtgtgcagccaaaatgccttgtacccgatgagtcctctgctccaagaatgcctccgggggtccaccaagtcctgtgctcgtacactcgtatccgggtcttttgggaaccggttcattttatcacaagggaacctaatagccaattgtgcatcaatcctttgcaagtgttacacaacaggaacgatcattaatcaagaccctgacaagatcctaacatacattgctgccgatcactgcccggtagtcgaggtgaacggcgtgaccatccaagtcgggagcaggaggtatccagacgctgtgtacttgcacagaattgacctcggtcctcccatatcattggagaggttggacgtagggacaaatctggggaatgcaattgctaagttggaggatgccaaggaattgttggagtcatcggaccagatattgaggagtatgaaaggtttatcgagcactagcatagtctacatcctgattgcagtgtgtcttggagggttgatagggatccccgctttaatatgttgctgcagggggcgttgtaacaaaaagggagaacaagttggtatgtcaagaccaggcctaaagcctgatcttacgggaacatcaaaatcctatgtaaggtcgctctgatcctctacaactcttgaaacacaaatgtcccacaagtctcctcttcgtcatcaagcaaccaccgcacccagcatcaagcccacctgaaattatctccggtttccctctggccgaacaatatcggtagttaattaaaacttagggtgcaagatcatccacaatgtcaccacaacgagaccggataaatgccttctacaaagataacccccatcccaagggaagtaggatagtcattaacagagaacatcttatgattgatagaccttatgttttgctggctgttctgtttgtcatgtttctgagcttgatcgggttgctagccattgcaggcattagacttcatcgggcagccatctacaccgcagagatccataaaagcctcagcaccaatctagatgtaactaactcaatcgagcatcaggtcaaggacgtgctgacaccactcttcaaaatcatcggtgatgaagtgggcctgaggacacctcagagattcactgacctagtgaaattcatctctgacaagattaaattccttaatccggatagggagtacgacttcagagatctcacttggtgtatcaacccgccagagagaatcaaattggattatgatcaatactgtgcagatgtggctgctgaagagctcatgaatgcattggtgaactcaactctactggagaccagaacaaccaatcagttcctagctgtctcaaagggaaactgctcagggcccactacaatcagaggtcaattctcaaacatgtcgctgtccctgttagacttgtatttaggtcgaggttacaatgtgtcatctatagtcactatgacatcccagggaatgtatgggggaacttacctagtggaaaagcctaatctgagcagcaaaaggtcagagttgtcacaactgagcatgtaccgagtgtttgaagtaggtgttatcagaaatccgggtttgggggctccggtgttccatatgacaaactatcttgagcaaccagtcagtaatgatctcagcaactgtatggtggctttgggggagctcaaactcgcagccctttgtcacggggaagattctatcacaattccctatcagggatcagggaaaggtgtcagcttccagctcgtcaagctaggtgtctggaaatccccaaccgacatgcaatcctgggtccccttatcaacggatgatccagtgatagacaggctttacctctcatctcacagaggtgttatcgctgacaaccaagcaaaatgggctgtcccgacaacacgaacagatgacaagttgcgaatggagacatgcttccaacaggcgtgtaagggtaaaatccaagcactctgcgagaatcccgagtgggcaccattgaaggataacaggattccttcatacggggtcttgtctgttgatctgagtctgacagttgagcttaaaatcaaaattgcttcgggattcgggccattgatcacacacggttcagggatggacctatacaaatccaaccacaacaatgtgtattggctgactatcccgccaatgaagaacctagccttaggtgtaatcaacacattggagtggataccgagattcaaggttagtccctacctcttcactgtcccaattaaggaagcaggcggagactgccatgccccaacatacctacctgcggaggtggatggtgatgtcaaactcagttccaatctggtgattctacctggtcaagatctccaatatgttttggcaacctacgatacttccagggttgaacatgctgtggtttattacgtttacagcccaagccgctcattttcttacttttatccttttaggttgcctataaagggggtccccatcgaattacaagtggaatgcttcacatgggaccaaaaactctggtgccgtcacttctgtgtgcttgcggactcagaatctggtggacatatcactcactctgggatggtgggcatgggagtcagctgcacagtcacccgggaagatggaaccaatcgcagatagggctgctagtgaaccaatcacatgatgtcacccagacatcaggcatacccactagtgtgaaatagacatcagaattaagaaaaacgtagggtccaagtggttccccgttatggactcgctatctgtcaaccagatcttataccctgaagttcacctagatagcccgatagttaccaataagatagtagccatcctggagtatgctcgagtccctcacgcttacagcctggaggaccctacactgtgtcagaacatcaagcaccgcctaaaaaacggattttccaaccaaatgattataaacaatgtggaagttgggaatgtcatcaagtccaagcttaggagttatccggcccactctcatattccatatccaaattgtaatcaggatttatttaacatagaagacaaagagtcaacgaggaagatccgtgaactcctcaaaaaggggaattcgctgtactccaaagtcagtgataaggttttccaatgcttaagggacactaactcacggcttggcctaggctccgaattgagggaggacatcaaggagaaagttattaacttgggagtttacatgcacagctcccagtggtttgagccctttctgttttggtttacagtcaagactgagatgaggtcagtgattaaatcacaaacccatacttgccataggaggagacacacacctgtattcttcactggtagttcagttgagttgctaatctctcgtgaccttgttgctataatcagtaaagagtctcaacatgtatattacctgacatttgaactggttttgatgtattgtgatgtcatagaggggaggttaatgacagagaccgctatgactattgatgctaggtatacagagcttctaggaagagtcagatacatgtggaaactgatagatggtttcttccctgcactcgggaatccaacttatcaaattgtagccatgctggagcctctttcacttgcttacctgcagctgagggatataacagtagaactcagaggtgctttccttaaccactgctttactgaaatacatgatgttcttgaccaaaacgggttttctgatgaaggtacttatcatgagttaattgaagctctagattacattttcataactgatgacatacatctgacaggggagattttctcatttttcagaagtttcggccaccccagacttgaagcagtaacggctgctgaaaatgttaggaaatacatgaatcagcctaaagtcattgtgtatgagactctgatgaaaggtcatgccatattttgtggaatcataatcaacggctatcgtgacaggcacggaggcagttggccaccgctgaccctccccctgcatgctgcagacacaatccggaatgctcaagcttcaggtgatgggttaacacatgagcagtgcgttgataactggaaatcttttgctggagtgaaatttggctgctttatgcctcttagcctggatagtgatctgacaatgtacctaaaggacaaggcacttgctgctctccaaagggaatgggattcagtttacccgaaagagttcctgcgttacgaccctcccaagggaaccgggtcacggaggcttgtagatgttttccttaatgattcgagctttgacccatatgatgtgataatgtatgttgtaagtggagcttacctccatgaccctgagttcaacctgtcttacagcctgaaagaaaaggagatcaaggaaacaggtagactttttgctaaaatgacttacaaaatgagggcatgccaagtgattgctgaaaatctaatctcaaacgggattggcaaatattttaaggacaatgggatggccaaggatgagcacgatttgactaaggcactccacactctagctgtctcaggagtccccaaagatctcaaagaaagtcacaggggggggccagtcttaaaaacctactcccgaagcccagtccacacaagtaccaggaacgtgagagcagcaaaagggtttatagggttccctcaagtaattcggcaggaccaagacactgatcatccggagaatatggaagcttacgagacagtcagtgcatttatcacgactgatctcaagaagtactgccttaattggagatatgagaccatcagcttgtttgcacagaggctaaatgagatttacggattgccctcatttttccagtggctgcataagaggcttgagacctctgtcctgtatgtaagtgaccctcattgcccccccgaccttgacgcccatatcccgttatataaagtccccaatgatcaaatcttcattaagtaccctatgggaggtatagaagggtattgtcagaagctgtggaccatcagcaccattccctatctatacctggctgcttatgagagcggagtaaggattgcttcgttagtgcaaggggacaatcagaccatagccgtaacaaaaagggtacccagcacatggccctacaaccttaagaaacgggaagctgctagagtaactagagattactttgtaattcttaggcaaaggctacatgatattggccatcacctcaaggcaaatgagacaattgtttcatcacatttttttgtctattcaaaaggaatatattatgatgggctacttgtgtcccaatcactcaagagcatcgcaagatgtgtattctggtcagagactatagttgatgaaacaagggcagcatgcagtaatattgctacaacaatggctaaaagcatcgagagaggttatgaccgttaccttgcatattccctgaacgtcctaaaagtgatacagcaaattctgatctctcttggcttcacaatcaattcaaccatgacccgggatgtagtcatacccctcctcacaaacaacgacctcttaataaggatggcactgttgcccgctcctattggggggatgaattatctgaatatgagcaggctgtttgtcagaaacatcggtgatccagtaacatcatcaattgctgatctcaagagaatgattctcgcctcactaatgcctgaagagaccctccatcaggtaatgacacaacaaccgggggactcttcattcctagactgggctagcgacccttactcagcaaatcttgtatgtgtccagagcatcactagactcctcaagaacataactgcaaggtttgtcctgatccatagtccaaacccaatgttaaaaggattattccatgatgacagtaaagaagaggacgagggactggcggcattcctcatggacaggcatattatagtacctagggcagctcatgaaatcctggatcatagtgtcacaggggcaagagagtctattgcaggcatgctggataccacaaaaggcttgattcgagccagcatgaggaaggggggtttaacctctcgagtgataaccagattgtccaattatgactatgaacaattcagagcagggatggtgctattgacaggaagaaagagaaatgtcctcattgacaaagagtcatgttcagtgcagctggcgagagctctaagaagccatatgtgggcgaggctagctcgaggacggcctatttacggccttgaggtccctgatgtactagaatctatgcgaggccaccttattcggcgtcatgagacatgtgtcatctgcgagtgtggatcagtcaactacggatggttttttgtcccctcgggttgccaactggatgatattgacaaggaaacatcatccttgagagtcccatatattggttctaccactgatgagagaacagacatgaagcttgccttcgtaagagccccaagtcgatccttgcgatctgctgttagaatagcaacagtgtactcatgggcttacggtgatgatgatagctcttggaacgaagcctggttgttggctaggcaaagggccaatgtgagcctggaggagctaagggtgatcactcccatctcaacttcgactaatttagcgcataggttgagggatcgtagcactcaagtgaaatactcaggtacatcccttgtccgagtggcgaggtataccacaatctccaacgacaatctctcatttgtcatatcagataagaaggttgatactaactttatataccaacaaggaatgcttctagggttgggtgttttagaaacattgtttcgactcgagaaagataccggatcatctaacacggtattacatcttcacgtcgaaacagattgttgcgtgatcccgatgatagatcatcccaggatacccagctcccgcaagctagagctgagggcagagctatgtaccaacccattgatatatgataatgcacctttaattgacagagatgcaacaaggctatacacccagagccataggaggcaccttgtggaatttgttacatggtccacaccccaactatatcacattttagctaagtccacagcactatctatgattgacctggtaacaaaatttgagaaggaccatatgaatgaaatttcagctctcataggggatgacgatatcaatagtttcataactgagtttctgctcatagagccaagattattcactatctacttgggccagtgtgcggccatcaattgggcatttgatgtacattatcatagaccatcagggaaatatcagatgggtgagctgttgtcatcgttcctttctagaatgagcaaaggagtgtttaaggtgcttgtcaatgctctaagccacccaaagatctacaagaaattctggcattgtggtattatagagcctatccatggtccttcacttgatgctcaaaacttgcacacaactgtgtgcaacatggtttacacatgctatatgacctacctcgacctgttgttgaatgaagagttagaagagttcacatttctcttgtgtgaaagcgacgaggatgtagtaccggacagattcgacaacatccaggcaaaacacttatgtgttctggcagatttgtactgtcaaccagggacctgcccaccaattcaaggtctaagaccggtagagaaatgtgcagttctaaccgaccatatcaaggcagaggctatgttatctccagcaggatcttcgtggaacataaatccaattattgtagaccattactcatgctccctgacttatctccggcgaggatcgatcaaacagataagattgagagttgatccaggattcattttcgacgccctcgctgaggtaaatgtcagtcagccaaagatcggcagcaacaacatctcaaatatgagcatcaaggctttcagacccccacacgatgatgttgcaaaattgctcaaagatatcaacacaagcaagcacaatcttcccatttcagggggcaatctcgccaattatgaaatccatgctttccgcagaatcgggttgaactcatctgcttgctacaaagctgttgagatatcaacattaattaggagatgccttgagccaggggaggacggcttgttcttgggtgagggatcgggttctatgttgatcacttataaggagatacttaaactaagcaagtgcttctataatagtggggtttccgccaattctagatctggtcaaagggaattagcaccctatccctccgaagttggccttgtcgaacacagaatgggagtaggtaatattgtcaaagtgctctttaacgggaggcccgaagtcacgtgggtaggcagtgtagattgcttcaatttcatagttagtaatatccctacctctagtgtggggtttatccattcagatatagagaccttgcctgacaaagatactatagagaagctagaggaattggcagccatcttatcgatggctctgctcctgggcaaaataggatcaatactggtgattaagcttatgcctttcagcggggattttgttcagggatttataagttatgtagggtctcattatagagaagtgaaccttgtataccctagatacagcaacttcatatctactgaatcttatttggttatgacagatctcaaggctaaccggctaatgaatcctgaaaagattaagcagcagataattgaatcatctgtgaggacttcacctggacttataggtcacatcctatccattaagcaactaagctgcatacaagcaattgtgggagacgcagttagtagaggtgatatcaatcctactctgaaaaaacttacacctatagagcaggtgctgatcaattgcgggttggcaattaacggacctaagctgtgcaaagaattgatccaccatgatgttgcctcagggcaagatggattgcttaattctatactcatcctctacagggagttggcaagattcaaagacaaccaaagaagtcaacaagggatgttccacgcttaccccgtattggtaagtagcaggcaacgagaacttatatctaggatcacccgcaaattttgggggcacattcttctttactccgggaacagaaagttgataaataagtttatccagaatctcaagtccggctatctgatactagacttacaccagaatatcttcgttaagaatctatccaagtcagagaaacagattattatgacggggggtttgaaacgtgagtgggtttttaaggtaacagtcaaggagaccaaagaatggtataagttagtcggatacagtgccctgattaaggactaattggttgaactccggaaccctaatcctgccctaggtggttaggcattatttgcaatatattaaagaaaactttgaaaatacgaagtttctattcccagctttgtctggt

SEQ ID NO: 4 - DNA, 3822 bp, Artificial Sequence
  Description of Artificial Sequence: Synthesized recombinant cDNA of SARS-CoV-2 spike protein
atgttcgtctttctggtgctccttcctctggtcagttctcagtgtgtgaatctcaccacaagaacccagttgcctcctgcttataccaacagctttacacggggtgtctattatcccgacaaggtgtttcgcagtagcgtactacactctacacaggacctttttctccccttcttctccaatgtcacttggtttcacgctatccacgtctcaggcacaaatggtaccaagcgctttgataatcccgttctgccctttaatgatggggtatattttgcctcaaccgaaaaatccaacatcatccggggatggatttttgggacaacccttgattccaagactcaaagcctgctgatcgttaacaatgctaccaacgttgtcatcaaagtatgcgagttccagttttgcaatgatccatttctcggcgtgtactaccataagaacaataaatcatggatggaatccgaattccgagtgtactcctctgctaacaactgcacctttgaatacgtatctcagccctttctcatggatctcgaaggaaagcagggaaatttcaagaacctccgggaatttgtcttcaagaatatagacgggtacttcaaaatctactctaagcatacccccatcaacctggtgcgcgacctaccacaaggcttcagtgccctagagcccctggtggacttgcccataggcattaatatcacgagatttcagacattattggccctgcacagaagctatctcacccctggcgattccagtagtggatggaccgctggcgcagccgcctattacgtgggatacttgcagccacgaactttcctactcaagtataatgagaacggaaccataaccgatgcagtagattgtgccttggatcctctttctgagacaaaatgtacactgaagtcgttcacagtggagaaagggatctaccagacaagcaacttcagggttcaaccgactgagtctatcgtcaggtttccaaatataaccaacctttgtccgtttggcgaagtgttcaatgccactagattcgcgtccgtctatgcatggaatcgcaaaaggatttccaactgtgtggccgattacagcgtgttgtacaattcagccagcttcagcacctttaagtgctatggagtgtctccaacgaaactcaacgatctgtgtttcacgaatgtgtacgccgattcattcgtcattcggggagacgaagtcagacagatagccccagggcagacagggaaaattgccgactataactacaaactgccagatgacttcaccggttgcgtgatagcttggaattctaataacctcgacagcaaggttggagggaactacaattatctgtaccggctgttccgtaagtcaaacctgaaaccctttgaacgcgacatctccacagagatttaccaagctggatccaccccttgcaatggggtagagggattcaattgctactttccgctgcagtcttatgggtttcaacccaccaatggagtggggtaccagccctaccgagtggttgtcctgtcctttgaattgttgcatgcccccgcgaccgtgtgtggccccaagaagagtacaaatctcgttaaaaacaagtgcgtaaacttcaactttaacggtttgacggggactggggtgctgacggaatcaaacaagaaattcctgccgttccagcagttcgggagggacattgccgacacaaccgacgctgtcagggatccacagaccctggagatcttggacattacaccttgctccttcggcggcgtgagtgtaatcacacctggaactaacacgagtaaccaggttgccgtcctgtaccaagacgtgaattgcaccgaggttccagttgcgatccacgcggatcagcttactcctacatggcgagtgtatagtacaggcagtaacgtattccagactcgtgccgggtgtttaataggggcagaacacgtgaataacagttatgagtgtgacattccgatcggcgctggtatatgcgcatcataccaaacccagactaactcacctagaagagcccgctccgtggccagccagagcattatcgcctatacgatgagcctgggtgctgagaattccgtagcatattctaacaattccattgctattcctaccaactttaccatctctgttaccactgagattctcccagtgtctatgactaagacatcagtggactgcactatgtatatctgcggcgatagcactgagtgtagcaatttgctcctgcaatatggttcattttgcacccagcttaatagggccctgacaggaattgccgttgagcaggacaagaatactcaggaggtcttcgctcaggttaagcagatctacaagactccgccaattaaggacttcggcggatttaacttcagccagattctgccagacccaagtaagccctccaaaaggtcttttatcgaggatctgctgttcaacaaagtgacacttgccgatgctggctttatcaaacagtatggagactgtctcggtgatatagcagcacgggacctcatctgcgcccagaagtttaacggactgaccgtcctgcctcctcttctgacagacgagatgattgctcagtacacttcggcgctgcttgcaggtactatcacaagcggctggacgtttggtgccggagccgcgctccaaattccattcgcaatgcagatggcttatagattcaacggcataggtgtcacccagaacgtgctgtacgaaaaccagaagctcatagcgaaccagtttaactccgccatagggaaaatccaggattcgctctccagtacagcatccgcattagggaaactgcaggacgttgtgaatcagaacgcccaagctcttaatacactggtgaaacaattgtcatccaatttcggggcaatcagctctgtgcttaatgacatcctctcacggctggataaagtcgaagccgaagttcagattgatcgcttgattactggtcggttacagtcactacagacatatgtgacccagcagctgattcgtgctgccgagattagggcatcggctaacctggcagctactaagatgtccgagtgcgtgcttggccaatcgaaacgcgtggatttctgtggcaaaggctatcatctgatgagcttccctcaaagcgcgccccatggcgtggtgtttctgcacgtgacgtatgtccccgcacaggagaagaatttcacaacagcccccgcaatctgtcacgatggcaaggcacactttcctcgagaaggggttttcgtgagcaatggcacccactggttcgtgacccagaggaacttttatgagccgcaaattatcactacggataatacctttgtgagtggaaactgtgacgtggtgattggaatcgtcaacaatactgtatacgaccccttacaacctgaactggactctttcaaagaggaactagacaagtactttaagaaccatacttctccagacgtcgatttaggagacatttcaggcatcaatgccagcgtggtgaacatccagaaggagatcgatagactgaacgaagtcgctaagaatttaaacgaaagcctaatagacctgcaagagctgggcaaatacgagcagtacattaagtggccatggtacatctggttgggcttcatcgctggccttatcgccattgttatggtcaccatcatgctctgctgcatgacttcttgttgcagttgcttaaaagggtgttgcagctgtggcagctgctgtaagttcgacgaggatgattccgagcccgtgctaaaaggtgttaagctgcattacacgtaa